European Patent Specification EP 2 650 305 B1, published May 8, 2024. Title: PC5 AS A FACTOR IX PROPEPTIDE PROCESSING ENZYME. Applicant: Biogen Idec Hemophilia Inc. Application Not yet assigned. The sequence listing filed with the application follows.

SEQUENCE LISTING (68 sequences)

SEQ ID NO: 1 - protein, 913 aa, Homo sapiens
  human PC5A
MGWGSRCCCPGRLDLLCVLALLGGCLLPVCRTRVYTNHWAVKIAGGFPEANRIASKYGFINIGQIGALKDYYHFYHSRTIKRSVISSRGTHSFISMEPKVEWIQQQVVKKRTKRDYDFSRAQSTYFNDPKWPSMWYMHCSDNTHPCQSDMNIEGAWKRGYTGKNIVVTILDDGIERTHPDLMQNYDALASCDVNGNDLDPMPRYDASNENKHGTRCAGEVAAAANNSHCTVGIAFNAKIGGVRMLDGDVTDMVEAKSVSFNPQHVHIYSASWGPDDDGKTVDGPAPLTRQAFENGVRMGRRGLGSVFVWASGNGGRSKDHCSCDGYTNSIYTISISSTAESGKKPWYLEECSSTLATTYSSGESYDKKIITTDLRQRCTDNHTGTSASAPMAAGIIALALEANPFLTWRDVQHVIVRTSRAGHLNANDWKTNAAGFKVSHLYGFGLMDAEAMVMEAEKWTTVPRQHVCVESTDRQIKTIRPNSAVRSIYKASGCSDNPNRHVNYLEHVVVRITITHPRRGDLAIYLTSPSGTRSQLLANRLFDHSMEGFKNWEFMTIHCWGERAAGDWVLEVYDTPSQLRNFKTPGKLKEWSLVLYGTSVQPYSPTNEFPKVERFRYSRVEDPTDDYGTEDYAGPCDPECSEVGCDGPGPDHCNDCLHYYYKLKNNTRICVSSCPPGHYHADKKRCRKCAPNCESCFGSHGDQCMSCKYGYFLNEETNSCVTHCPDGSYQDTKKNLCRKCSENCKTCTEFHNCTECRDGLSLQGSRCSVSCEDGRYFNGQDCQPCHRFCATCAGAGADGCINCTEGYFMEDGRCVQSCSISYYFDHSSENGYKSCKKCDISCLTCNGPGFKNCTSCPSGYLLDLGMCQMGAICKDATEESWAEGGFCMLVKKNNLCQRKVLQQLCCKTCTFQG

SEQ ID NO: 2 - DNA, 2739 bp, Homo sapiens
  human PC5A
atgggctgggggagccgctgctgctgcccgggacgtttggacctgctgtgcgtgctggcgctgctcgggggctgcctgctccccgtgtgtcggacgcgcgtctacaccaaccactgggcagtcaaaatcgccgggggcttcccggaggccaaccgtatcgccagcaagtacggattcatcaacataggacagataggggccctgaaggactactaccacttctaccatagcaggacgattaaaaggtcagttatctcgagcagagggacccacagtttcatttcaatggaaccaaaggtggaatggatccaacagcaagtggtaaaaaagcggacaaagagggattatgacttcagtcgtgcccagtctacctatttcaatgatcccaagtggcccagcatgtggtatatgcactgcagtgacaatacacatccctgccagtctgacatgaatatcgaaggagcctggaagagaggctacacgggaaagaacattgtggtcactatcctggatgacggaattgagagaacccatccagatctgatgcaaaactacgatgctctggcaagttgcgacgtgaatgggaatgacttggacccaatgcctcgttatgatgcaagcaacgagaacaagcatgggactcgctgtgctggagaagtggcagccgctgcaaacaattcgcactgcacagtcggaattgctttcaacgccaagatcggaggagtgcgaatgctggacggagatgtcacggacatggttgaagcaaaatcagttagcttcaacccccagcacgtgcacatttacagcgccagctggggcccggatgatgatggcaagactgtggacggaccagcccccctcacccggcaagcctttgaaaacggcgttagaatggggcggagaggcctcggctctgtgtttgtttgggcatctggaaatggtggaaggagcaaagaccactgctcctgtgatggctacaccaacagcatctacaccatctccatcagcagcactgcagaaagcggaaagaaaccttggtacctggaagagtgttcatccacgctggccacaacctacagcagcggggagtcctacgataagaaaatcatcactacagatctgaggcagcgttgcacggacaaccacactgggacgtcagcctcagcccccatggctgcaggcatcattgcgctggccctggaagccaatccgtttctgacctggagagacgtacagcatgttattgtcaggacttcccgtgcgggacatttgaacgctaatgactggaaaaccaatgctgctggttttaaggtgagccatctttatggatttggactgatggacgcagaagccatggtgatggaggcagagaagtggaccaccgttccccggcagcacgtgtgtgtggagagcacagaccgacaaatcaagacaatccgccctaacagtgcagtgcgctccatctacaaagcttcaggctgctcggataaccccaaccgccatgtcaactacctggagcacgtcgttgtgcgcatcaccatcacccaccccaggagaggagacctggccatctacctgacctcgccctctggaactaggtctcagcttttggccaacaggctatttgatcactccatggaaggattcaaaaactgggagttcatgaccattcattgctggggagaaagagctgctggtgactgggtccttgaagtttatgatactccctctcagctaaggaactttaagactccaggtaaattgaaagaatggtctttggtcctctacggcacctccgtgcagccatattcaccaaccaatgaatttccgaaagtggaacggttccgctatagccgagttgaagaccccacagacgactatggcacagaggattatgcaggtccctgcgaccctgagtgcagtgaggttggctgtgacgggccaggaccagaccactgcaatgactgtttgcactactactacaagctgaaaaacaataccaggatctgtgtctccagctgcccccctggccactaccacgccgacaagaagcgctgcaggaagtgtgcccccaactgtgagtcctgctttgggagccatggtgaccaatgcatgtcctgcaaatatggatactttctgaatgaagaaaccaacagctgtgttactcactgccctgatgggtcatatcaggataccaagaaaaatctttgccggaaatgcagtgaaaactgcaagacatgtactgaattccataactgtacagaatgtagggatgggttaagcctgcagggatcccggtgctctgtctcctgtgaagatggacggtatttcaacggccaggactgccagccctgccaccgcttctgcgccacttgtgctggggcaggagctgatgggtgcattaactgcacagagggctacttcatggaggatgggagatgcgtgcagagctgtagtatcagctattactttgaccactcttcagagaatggatacaaatcctgcaaaaaatgtgatatcagttgtttgacgtgcaatggcccaggattcaagaactgtacaagctgccctagtgggtatctcttagacttaggaatgtgtcaaatgggagccatttgcaaggatgcaacggaagagtcctgggcggaaggaggcttctgtatgcttgtgaaaaagaacaatctgtgccaacggaaggttcttcaacaactttgctgcaaaacatgtacatttcaaggc

SEQ ID NO: 3 - protein, 461 aa, Homo sapiens
  human factor IX proprotein
MQRVNMIMAESPGLITICLLGYLLSAECTVFLDHENANKILNRPKRYNSGKLEEFVQGNLERECMEEKCSFEEAREVFENTERTTEFWKQYVDGDQCESNPCLNGGSCKDDINSYECWCPFGFEGKNCELDVTCNIKNGRCEQFCKNSADNKVVCSCTEGYRLAENQKSCEPAVPFPCGRVSVSQTSKLTRAETVFPDVDYVNSTEAETILDNITQSTQSFNDFTRVVGGEDAKPGQFPWQVVLNGKVDAFCGGSIVNEKWIVTAAHCVETGVKITVVAGEHNIEETEHTEQKRNVIRIIPHHNYNAAINKYNHDIALLELDEPLVLNSYVTPICIADKEYTNIFLKFGSGYVSGWGRVFHKGRSALVLQYLRVPLVDRATCLRSTKFTIYNNMFCAGFHEGGRDSCQGDSGGPHVTEVEGTSFLTGIISWGEECAMKGKYGIYTKVSRYVNWIKEKTKLT

SEQ ID NO: 4 - DNA, 1383 bp, Homo sapiens
  human factor IX proprotein
atgcagcgcgtgaacatgatcatggcagaatcaccaggcctcatcaccatctgccttttaggatatctactcagtgctgaatgtacagtttttcttgatcatgaaaacgccaacaaaattctgaatcggccaaagaggtataattcaggtaaattggaagagtttgttcaagggaaccttgagagagaatgtatggaagaaaagtgtagttttgaagaagcacgagaagtttttgaaaacactgaaagaacaactgaattttggaagcagtatgttgatggagatcagtgtgagtccaatccatgtttaaatggcggcagttgcaaggatgacattaattcctatgaatgttggtgtccctttggatttgaaggaaagaactgtgaattagatgtaacatgtaacattaagaatggcagatgcgagcagttttgtaaaaatagtgctgataacaaggtggtttgctcctgtactgagggatatcgacttgcagaaaaccagaagtcctgtgaaccagcagtgccatttccatgtggaagagtttctgtttcacaaacttctaagctcacccgtgctgagactgtttttcctgatgtggactatgtaaattctactgaagctgaaaccattttggataacatcactcaaagcacccaatcatttaatgacttcactcgggttgttggtggagaagatgccaaaccaggtcaattcccttggcaggttgttttgaatggtaaagttgatgcattctgtggaggctctatcgttaatgaaaaatggattgtaactgctgcccactgtgttgaaactggtgttaaaattacagttgtcgcaggtgaacataatattgaggagacagaacatacagagcaaaagcgaaatgtgattcgaattattcctcaccacaactacaatgcagctattaataagtacaaccatgacattgcccttctggaactggacgaacccttagtgctaaacagctacgttacacctatttgcattgctgacaaggaatacacgaacatcttcctcaaatttggatctggctatgtaagtggctggggaagagtcttccacaaagggagatcagctttagttcttcagtaccttagagttccacttgttgaccgagccacatgtcttcgatctacaaagttcaccatctataacaacatgttctgtgctggcttccatgaaggaggtagagattcatgtcaaggagatagtgggggaccccatgttactgaagtggaagggaccagtttcttaactggaattattagctggggtgaagagtgtgcaatgaaaggcaaatatggaatatataccaaggtatcccggtatgtcaactggattaaggaaaaaacaaagctcact

SEQ ID NO: 5 - protein, 227 aa, Homo sapiens
  human Fc gamma
DKTHTCPPCPAPELLGGPSVFLFPPKPKDTLMISRTPEVTCVVVDVSHEDPEVKFNWYVDGVEVHNAKTKPREEQYNSTYRVVSVLTVLHQDWLNGKEYKCKVSNKALPAPIEKTISKAKGQPREPQVYTLPPSRDELTKNQVSLTCLVKGFYPSDIAVEWESNGQPENNYKTTPPVLDSDGSFFLYSKLTVDKSRWQQGNVFSCSVMHEALHNHYTQKSLSLSPGK

SEQ ID NO: 6 - protein, 4 aa, Homo sapiens
ELLG

SEQ ID NO: 7 - protein, 8 aa, Artificial sequence
  synthetic peptide
EFAGAAAV

SEQ ID NO: 8 - protein, 10 aa, Artificial sequence
  synthetic peptide; with respect to position 2-10 any one or more Gly units may be absent
GGGGGGGGGG

SEQ ID NO: 9 - protein, 20 aa, Artificial sequence
  synthetic peptide; with respect to position 3-20 any one or more Gly-Ala units may be absent
GAGAGAGAGAGAGAGAGAGA

SEQ ID NO: 10 - protein, 30 aa, Artificial sequence
  synthetic peptide; with respect to position 4-30 any one or more Gly-Gly-Ser units may be absent
GGSGGSGGSGGSGGSGGSGGSGGSGGSGGS

SEQ ID NO: 11 - protein, 50 aa, Artificial sequence
  synthetic peptide; with respect to position 6-50 any one or more Gly-Gly-Gly-Gly-Ser units may be absent
GGGGSGGGGSGGGGSGGGGSGGGGSGGGGSGGGGSGGGGSGGGGSGGGGS

SEQ ID NO: 12 - protein, 7 aa, Artificial sequence
  synthetic peptide
SGGSGGS

SEQ ID NO: 13 - protein, 15 aa, Artificial sequence
  synthetic peptide
GGSGGSGGSGGSGGG

SEQ ID NO: 14 - protein, 16 aa, Artificial sequence
  synthetic peptide
GGSGGSGGGGSGGGGS

SEQ ID NO: 15 - protein, 18 aa, Artificial sequence
  synthetic peptide
GGSGGSGGSGGSGGSGGS

SEQ ID NO: 16 - protein, 30 aa, Artificial sequence
  synthetic peptide
GGGGSGGGGSGGGGSGGGGSGGGGSGGGGS

SEQ ID NO: 17 - protein, 18 aa, Homo sapiens
TVFLDHENANKILNRPKR

SEQ ID NO: 18 - protein, 11 aa, Homo sapiens
TVFLDHENANK

SEQ ID NO: 19 - protein, 6 aa, Homo sapiens
YGIYTK

SEQ ID NO: 20 - DNA, 69 bp, Artificial sequence
  synthetic oligonucleotide
gctgcggtcgacaaaactcacacatgcccaccgtgcccagctccggaactcctgggcggaccgtcagtc

SEQ ID NO: 21 - DNA, 36 bp, Artificial sequence
  synthetic oligonucleotide
attggaattctcatttacccggagacagggagaggc

SEQ ID NO: 22 - DNA, 102 bp, Artificial sequence
  synthetic oligonucleotide
tttaagcttgccgccaccatggagacagacacactcctgctatgggtactgctgctctgggttccaggttccactggtgacaaaactcacacatgcccaccg

SEQ ID NO: 23 - DNA, 22 bp, Artificial sequence
  synthetic oligonucleotide
ggtcagctcatcgcgggatggg

SEQ ID NO: 24 - DNA, 22 bp, Artificial sequence
  synthetic oligonucleotide
cccatcccgcgatgagctgacc

SEQ ID NO: 25 - DNA, 9 bp, Artificial sequence
  synthetic oligonucleotide
gccgccacc

SEQ ID NO: 26 - DNA, 33 bp, Artificial sequence
  synthetic oligonucleotide
ttactgcagaaggttatgcagcgcgtgaacatg

SEQ ID NO: 27 - DNA, 26 bp, Artificial sequence
  synthetic oligonucleotide
agtgagctttgttttttccttaatcc

SEQ ID NO: 28 - DNA, 38 bp, Artificial sequence
  synthetic oligonucleotide
caagggaatctagagagagaatgtatggaagaaaagtg

SEQ ID NO: 29 - DNA, 37 bp, Artificial sequence
  synthetic oligonucleotide
acattctctctctagattcccttgaacaaactcttcc

SEQ ID NO: 30 - DNA, 24 bp, Artificial sequence
  synthetic oligonucleotide
atgacatccactttgcctttctct

SEQ ID NO: 31 - DNA, 20 bp, Artificial sequence
  synthetic oligonucleotide
atagaagcctttgaccaggc

SEQ ID NO: 32 - DNA, 39 bp, Artificial sequence
  synthetic oligonucleotide
aaaaacaaagctcactgacaaaactcacacatgcccacc

SEQ ID NO: 33 - DNA, 42 bp, Artificial sequence
  synthetic oligonucleotide
gtgtgagttttgtcagtgagctttgttttttccttaatccag

SEQ ID NO: 34 - DNA, 37 bp, Artificial sequence
  synthetic oligonucleotide
atgcggccgcgccgccaccatggagacagacacactc

SEQ ID NO: 35 - DNA, 26 bp, Artificial sequence
  synthetic oligonucleotide
atctcgagtcatttacccggagacag

SEQ ID NO: 36 - DNA, 51 bp, Artificial sequence
  synthetic oligonucleotide
gtcaaagcttcgcgacgtacggccgccaccatgcagcgcgtgaacatgatc

SEQ ID NO: 37 - DNA, 35 bp, Artificial sequence
  synthetic oligonucleotide
ctgtgatgttcccacagtacttaccaacctgcgtg

SEQ ID NO: 38 - DNA, 21 bp, Artificial sequence
  synthetic oligonucleotide
agtactgtgggaacatcacag

SEQ ID NO: 39 - DNA, 33 bp, Artificial sequence
  synthetic oligonucleotide
tgactctagattcccttgaacaaactcttccaa

SEQ ID NO: 40 - DNA, 24 bp, Artificial sequence
  synthetic oligonucleotide
atctacaccatctccatcagcagc

SEQ ID NO: 41 - DNA, 37 bp, Artificial sequence
  synthetic oligonucleotide
aaggcggccgctcagccttgaaatgtacatgttttgc

SEQ ID NO: 42 - DNA, 18 bp, Artificial sequence
  synthetic oligonucleotide
agcgagggagcagcgagg

SEQ ID NO: 43 - DNA, 21 bp, Artificial sequence
  synthetic oligonucleotide
ggtagttgacatggcggttgg

SEQ ID NO: 44 - DNA, 34 bp, Artificial sequence
  synthetic oligonucleotide
cagcgacttaagccaccatgggctgggggagccg

SEQ ID NO: 45 - DNA, 20 bp, Artificial sequence
  synthetic oligonucleotide
gtaggttgtggccagcgtgg

SEQ ID NO: 46 - DNA, 34 bp, Artificial sequence
  synthetic oligonucleotide
ggtaagcttgccatggagctgaggccctggttgc

SEQ ID NO: 47 - DNA, 27 bp, Artificial sequence
  synthetic oligonucleotide
gttttcaatctctaggacccactcgcc

SEQ ID NO: 48 - DNA, 23 bp, Artificial sequence
  synthetic oligonucleotide
gccaggccacatgactactccgc

SEQ ID NO: 49 - DNA, 34 bp, Artificial sequence
  synthetic oligonucleotide
ggtgaattctcactcaggcaggtgtgagggcagc

SEQ ID NO: 50 - DNA, 53 bp, Artificial sequence
  synthetic oligonucleotide
gcgctagccgtacggccgccaccatgaaagtgaggaaatatattactttatgc

SEQ ID NO: 51 - DNA, 29 bp, Artificial sequence
  synthetic oligonucleotide
gctattgatcacaaagatctacatcctcc

SEQ ID NO: 52 - DNA, 29 bp, Artificial sequence
  synthetic oligonucleotide
ggaggatgtagatctttgtgatcaatagc

SEQ ID NO: 53 - DNA, 59 bp, Artificial sequence
  synthetic oligonucleotide
gcgaattccggtccgtcattgcctagggctcgagagttttttaggagtgtttggatcag

SEQ ID NO: 54 - DNA, 21 bp, Artificial sequence
  synthetic oligonucleotide
gcatggactccgatcccaacg

SEQ ID NO: 55 - DNA, 21 bp, Artificial sequence
  synthetic oligonucleotide
cgttgggatcggagtccatgc

SEQ ID NO: 56 - DNA, 40 bp, Artificial sequence
  synthetic oligonucleotide
ggtaagcttgccgccaccatgccgaaggggaggcagaaag

SEQ ID NO: 57 - DNA, 33 bp, Artificial sequence
  synthetic oligonucleotide
tttgaattctcagttgggggtgatggtgtaacc

SEQ ID NO: 58 - DNA, 20 bp, Artificial sequence
  synthetic oligonucleotide
ggcacctgaataaccgacgg

SEQ ID NO: 59 - DNA, 20 bp, Artificial sequence
  synthetic oligonucleotide
cgtcacgttgatgtccctgc

SEQ ID NO: 60 - protein, 19 aa, Artificial sequence
  synthetic peptide
TVFLDHENANKILNRPKRC

SEQ ID NO: 61 - DNA, 2739 bp, Artificial sequence
  synthetic oligonucleotide
atgggctgggggagccgctgctgctgcccgggacgtttggacctgctgtgcgtgctggcgctgctcgggggctgcctgctccccgtgtgtcggacgcgcgtctacaccaaccactgggcagtcaaaatcgccgggggcttcccggaggccaaccgtatcgccagcaagtacggattcatcaacataggacagataggggccctgaaggactactaccacttctaccatagcaggacgattaaaaggtcagttatctcgagcagagggacccacagtttcatttcaatggaaccaaaggtggaatggatccaacagcaagtggtaaaaaagcggacaaagagggattatgacttcagtcgtgcccagtctacctatttcaatgatcccaagtggcccagtatgtggtatatgcactgcagtgacaatacacatccctgccagtctgacatgaatatcgaaggagcctggaagagaggctacacgggaaagaacattgtggtcactatcctggatgacggaattgagagaacccatccagatctgatgcaaaactacgatgctctggcaagttgcgacgtgaatgggaatgacttggacccaatgcctcgttatgatgcaagcaacgagaacaagcatgggactcgctgtgctggagaagtggcagccgctgcaaacaattcgcactgcacagtcggaattgctttcaacgccaagatcggaggagtgcgaatgctggacggagatgtcacggacatggttgaagcaaaatcagttagcttcaacccccagcacgtgcacatttacagcgccagctggggcccggatgatgatggcaagactgtggacggaccagcccccctcacccggcaagcctttgaaaacggcgttagaatggggcggagaggcctcggctctgtgtttgtttgggcatctggaaatggtggaaggagcaaagaccactgctcctgtgatggctacaccaacagcatctacaccatctccatcagcagcactgcagaaagcggaaagaaaccttggtacctggaagagtgttcatccacgctggccacaacctacagcagcggggagtcctacgataagaaaatcatcactacagatctgaggcagcgttgcacggacaaccacactgggacgtcagcctcagcccccatggctgcaggcatcattgcgctggccctggaagccaatccgtttctgacctggagagacgtacagcatgttattgtcaggacttcccgtgcgggacatttgaacgctaatgactggaaaaccaatgctgctggttttaaggtgagccatctttatggatttggactgatggacgcagaagccatggtgatggaggcagagaagtggaccaccgttccccggcagcacgtgtgtgtggagagcacagaccgacaaatcaagacaatccgccctaacagtgcagtgcgctccatctacaaagcctcaggctgctcagataaccccaaccgccatgtcaactacctggagcacgtcgttgtgcgcatcaccatcacccaccccaggagaggagacctggccatctacctgacctcgccctctggaactaggtctcagcttttggccaacaggctatttgatcactccatggaaggattcaaaaactgggagttcatgaccattcattgctggggagaaagagctgctggtgactgggtccttgaagtttatgatactccctctcagctaaggaactttaagactccaggtaaattgaaagaatggtctttggtcctctacggcacctccgtgcagccatattcaccaaccaatgaatttccgaaagtggaacggttccgctatagccgagttgaagaccccacagacgactatggcacagaggattatgcaggtccctgcgaccctgagtgcagtgaggttggctgtgacgggccaggaccagaccactgcaatgactgtttgcactactactacaagctgaaaaacaataccaggatctgtgtctccagctgcccccctggccactaccacgccgacaagaagcgctgcaggaagtgtgcccccaactgtgagtcctgctttgggagccatggtgaccaatgcatgtcctgcaaatatggatactttctgaatgaagaaaccaacagctgtgttactcactgccctgatgggtcatatcaggataccaagaaaaatctttgccggaaatgcagtgaaaactgcaagacatgtactgaattccataactgtacagaatgtagggatgggttaagcctgcagggatcccggtgctctgtctcctgtgaagatggacggtatttcaacggccaggactgccagccctgccaccgcttctgcgccacttgtgctggggcaggagctgatgggtgcattaactgcacagagggctacttcatggaggatgggagatgcgtgcagagctgtagtatcagctattactttgaccactcttcagagaatggatacaaatcctgcaaaaaatgtgatatcagttgtttgacgtgcaatggcccaggattcaagaactgtacaagctgccctagtgggtatctcttagacttaggaatgtgtcaaatgggagccatttgcaaggatgcaacggaagagtcctgggcggaaggaggcttctgtatgcttgtgaaaaagaacaatctgtgccaacggaaggttcttcaacaactttgctgcaaaacatgtacatttcaaggc

SEQ ID NO: 62 - DNA, 681 bp, Homo sapiens
  human Fc gamma 1
gacaaaactcacacatgcccaccgtgcccagcacctgaactcctggggggaccgtcagtcttcctcttccccccaaaacccaaggacaccctcatgatctcccggacccctgaggtcacatgcgtggtggtggacgtgagccacgaagaccctgaggtcaagttcaactggtacgtggacggcgtggaggtgcataatgccaagacaaagccgcgggaggagcagtacaacagcacgtaccgtgtggtcagcgtcctcaccgtcctgcaccaggactggctgaatggcaaggagtacaagtgcaaggtctccaacaaagccctcccagcccccatcgagaaaaccatctccaaagccaaagggcagccccgagaaccacaggtgtacaccctgcccccatcccgggatgagctgaccaagaaccaggtcagcctgacctgcctggtcaaaggcttctatcccagcgacatcgccgtggagtgggagagcaatgggcagccggagaacaactacaagaccacgcctcccgtgctggactccgacggctccttcttcctctacagcaagctcaccgtggacaagagcaggtggcagcaggggaacgtcttctcatgctccgtgatgcatgaggctctgcacaaccactacacgcagaagagcctctccctgtctccgggtaaa

SEQ ID NO: 63 - DNA, 741 bp, Artificial sequence
  synthetic oligonucleotide
atggagacagacacactcctgctatgggtactgctgctctgggttccaggttccactggtgacaaaactcacacatgcccaccgtgcccagctccggaactgctgggcggaccgtcagtcttcctcttccccccaaaacccaaggacaccctcatgatctcccggacccctgaggtcacatgcgtggtggtggacgtgagccacgaagaccctgaggtcaagttcaactggtacgtggacggcgtggaggtgcataatgccaagacaaagccgcgggaggagcagtacaacagcacgtaccgtgtggtcagcgtcctcaccgtcctgcaccaggactggctgaatggcaaggagtacaagtgcaaggtctccaacaaagccctcccagcccccatcgagaaaaccatctccaaagccaaagggcagccccgagaaccacaggtgtacaccctgcccccatcccgcgatgagctgaccaagaaccaggtcagcctgacctgcctggtcaaaggcttctatcccagcgacatcgccgtggagtgggagagcaatgggcagccggagaacaactacaagaccacgcctcccgtgttggactccgacggctccttcttcctctacagcaagctcaccgtggacaagagcaggtggcagcaggggaacgtcttctcatgctccgtgatgcatgaggctctgcacaaccactacacgcagaagagcctctccctgtctccgggtaaa

SEQ ID NO: 64 - protein, 247 aa, Artificial sequence
  synthetic peptide
METDTLLLWVLLLWVPGSTGDKTHTCPPCPAPELLGGPSVFLFPPKPKDTLMISRTPEVTCVVVDVSHEDPEVKFNWYVDGVEVHNAKTKPREEQYNSTYRVVSVLTVLHQDWLNGKEYKCKVSNKALPAPIEKTISKAKGQPREPQVYTLPPSRDELTKNQVSLTCLVKGFYPSDIAVEWESNGQPENNYKTTPPVLDSDGSFFLYSKLTVDKSRWQQGNVFSCSVMHEALHNHYTQKSLSLSPGK

SEQ ID NO: 65 - DNA, 2064 bp, Artificial sequence
  synthetic oligonucleotide; FIX-Fc
atgcagcgcgtgaacatgatcatggcagaatcaccaggcctcatcaccatctgccttttaggatatctactcagtgctgaatgtacagtttttcttgatcatgaaaacgccaacaaaattctgaatcggccaaagaggtataattcaggtaaattggaagagtttgttcaagggaatctagagagagaatgtatggaagaaaagtgtagttttgaagaagcacgagaagtttttgaaaacactgaaagaacaactgaattttggaagcagtatgttgatggagatcagtgtgagtccaatccatgtttaaatggcggcagttgcaaggatgacattaattcctatgaatgttggtgtccctttggatttgaaggaaagaactgtgaattagatgtaacatgtaacattaagaatggcagatgcgagcagttttgtaaaaatagtgctgataacaaggtggtttgctcctgtactgagggatatcgacttgcagaaaaccagaagtcctgtgaaccagcagtgccatttccatgtggaagagtttctgtttcacaaacttctaagctcacccgtgctgagactgtttttcctgatgtggactatgtaaattctactgaagctgaaaccattttggataacatcactcaaagcacccaatcatttaatgacttcactcgggttgttggtggagaagatgccaaaccaggtcaattcccttggcaggttgttttgaatggtaaagttgatgcattctgtggaggctctatcgttaatgaaaaatggattgtaactgctgcccactgtgttgaaactggtgttaaaattacagttgtcgcaggtgaacataatattgaggagacagaacatacagagcaaaagcgaaatgtgattcgaattattcctcaccacaactacaatgcagctattaataagtacaaccatgacattgcccttctggaactggacgaacccttagtgctaaacagctacgttacacctatttgcattgctgacaaggaatacacgaacatcttcctcaaatttggatctggctatgtaagtggctggggaagagtcttccacaaagggagatcagctttagttcttcagtaccttagagttccacttgttgaccgagccacatgtcttcgatctacaaagttcaccatctataacaacatgttctgtgctggcttccatgaaggaggtagagattcatgtcaaggagatagtgggggaccccatgttactgaagtggaagggaccagtttcttaactggaattattagctggggtgaagagtgtgcaatgaaaggcaaatatggaatatataccaaggtgtcccggtatgtcaactggattaaggaaaaaacaaagctcactgacaaaactcacacatgcccaccgtgcccagctccggaactcctgggcggaccgtcagtcttcctcttccccccaaaacccaaggacaccctcatgatctcccggacccctgaggtcacatgcgtggtggtggacgtgagccacgaagaccctgaggtcaagttcaactggtacgtggacggcgtggaggtgcataatgccaagacaaagccgcgggaggagcagtacaacagcacgtaccgtgtggtcagcgtcctcaccgtcctgcaccaggactggctgaatggcaaggagtacaagtgcaaggtctccaacaaagccctcccagcccccatcgagaaaaccatctccaaagccaaagggcagccccgagaaccacaggtgtacaccctgcccccatcccgggatgagctgaccaagaaccaggtcagcctgacctgcctggtcaaaggcttctatcccagcgacatcgccgtggagtgggagagcaatgggcagccggagaacaactacaagaccacgcctcccgtgttggactccgacggctccttcttcctctacagcaagctcaccgtggacaagagcaggtggcagcaggggaacgtcttctcatgctccgtgatgcatgaggctctgcacaaccactacacgcagaagagcctctccctgtctccgggtaaa

SEQ ID NO: 66 - protein, 688 aa, artificial sequence
  synthetic peptide
MQRVNMIMAESPGLITICLLGYLLSAECTVFLDHENANKILNRPKRYNSGKLEEFVQGNLERECMEEKCSFEEAREVFENTERTTEFWKQYVDGDQCESNPCLNGGSCKDDINSYECWCPFGFEGKNCELDVTCNIKNGRCEQFCKNSADNKVVCSCTEGYRLAENQKSCEPAVPFPCGRVSVSQTSKLTRAETVFPDVDYVNSTEAETILDNITQSTQSFNDFTRVVGGEDAKPGQFPWQVVLNGKVDAFCGGSIVNEKWIVTAAHCVETGVKITVVAGEHNIEETEHTEQKRNVIRIIPHHNYNAAINKYNHDIALLELDEPLVLNSYVTPICIADKEYTNIFLKFGSGYVSGWGRVFHKGRSALVLQYLRVPLVDRATCLRSTKFTIYNNMFCAGFHEGGRDSCQGDSGGPHVTEVEGTSFLTGIISWGEECAMKGKYGIYTKVSRYVNWIKEKTKLTDKTHTCPPCPAPELLGGPSVFLFPPKPKDTLMISRTPEVTCVVVDVSHEDPEVKFNWYVDGVEVHNAKTKPREEQYNSTYRVVSVLTVLHQDWLNGKEYKCKVSNKALPAPIEKTISKAKGQPREPQVYTLPPSRDELTKNQVSLTCLVKGFYPSDIAVEWESNGQPENNYKTTPPVLDSDGSFFLYSKLTVDKSRWQQGNVFSCSVMHEALHNHYTQKSLSLSPGK

SEQ ID NO: 67 - DNA, 741 bp, Artificial sequence
  synthetic oligonucleotide
atggagacagacacactcctgctatgggtactgctgctctgggttccaggttccactggtgacaaaactcacacatgcccaccgtgcccagcacctgaactcctgggaggaccgtcagtcttcctcttccccccaaaacccaaggacaccctcatgatctcccggacccctgaggtcacatgcgtggtggtggacgtgagccacgaagaccctgaggtcaagttcaactggtacgtggacggcgtggaggtgcataatgccaagacaaagccgcgggaggagcagtacaacagcacgtaccgtgtggtcagcgtcctcaccgtcctgcaccaggactggctgaatggcaaggagtacaagtgcaaggtctccaacaaagccctcccagcccccatcgagaaaaccatctccaaagccaaagggcagccccgagaaccacaggtgtacaccctgcccccatcccgcgatgagctgaccaagaaccaggtcagcctgacctgcctggtcaaaggcttctatcccagcgacatcgccgtggagtgggagagcaatgggcagccggagaacaactacaagaccacgcctcccgtgttggactccgacggctccttcttcctctacagcaagctcaccgtggacaagagcaggtggcagcaggggaacgtcttctcatgctccgtgatgcatgaggctctgcacaaccactacacgcagaagagcctctccctgtctccgggtaaa

SEQ ID NO: 68 - DNA, 2363 bp, Artificial sequence
  synthetic oligonucleotide; FIX-Fc
atgcagcgcgtgaacatgatcatggcagaatcaccaggcctcatcaccatctgccttttaggatatctactcagtgctgaatgtacaggtttgtttccttttttaaaatacattgagtatgcttgccttttagatatagaaatatctgatgctgtcttcttcactaaattttgattacatgatttgacagcaatattgaagagtctaacagccagcacgcaggttggtaagtactgtgggaacatcacagattttggctccatgccctaaagagaaattggctttcagattatttggattaaaaacaaagactttcttaagagatgtaaaattttcatgatgttttcttttttgctaaaactaaagaattattcttttacatttcagtttttcttgatcatgaaaacgccaacaaaattctgaatcggccaaagaggtataattcaggtaaattggaagagtttgttcaagggaatctagagagagaatgtatggaagaaaagtgtagttttgaagaagcacgagaagtttttgaaaacactgaaagaacaactgaattttggaagcagtatgttgatggagatcagtgtgagtccaatccatgtttaaatggcggcagttgcaaggatgacattaattcctatgaatgttggtgtccctttggatttgaaggaaagaactgtgaattagatgtaacatgtaacattaagaatggcagatgcgagcagttttgtaaaaatagtgctgataacaaggtggtttgctcctgtactgagggatatcgacttgcagaaaaccagaagtcctgtgaaccagcagtgccatttccatgtggaagagtttctgtttcacaaacttctaagctcacccgtgctgagactgtttttcctgatgtggactatgtaaattctactgaagctgaaaccattttggataacatcactcaaagcacccaatcatttaatgacttcactcgggttgttggtggagaagatgccaaaccaggtcaattcccttggcaggttgttttgaatggtaaagttgatgcattctgtggaggctctatcgttaatgaaaaatggattgtaactgctgcccactgtgttgaaactggtgttaaaattacagttgtcgcaggtgaacataatattgaggagacagaacatacagagcaaaagcgaaatgtgattcgaattattcctcaccacaactacaatgcagctattaataagtacaaccatgacattgcccttctggaactggacgaacccttagtgctaaacagctacgttacacctatttgcattgctgacaaggaatacacgaacatcttcctcaaatttggatctggctatgtaagtggctggggaagagtcttccacaaagggagatcagctttagttcttcagtaccttagagttccacttgttgaccgagccacatgtcttcgatctacaaagttcaccatctataacaacatgttctgtgctggcttccatgaaggaggtagagattcatgtcaaggagatagtgggggaccccatgttactgaagtggaagggaccagtttcttaactggaattattagctggggtgaagagtgtgcaatgaaaggcaaatatggaatatataccaaggtgtcccggtatgtcaactggattaaggaaaaaacaaagctcactgacaaaactcacacatgcccaccgtgcccagctccggaactcctgggcggaccgtcagtcttcctcttccccccaaaacccaaggacaccctcatgatctcccggacccctgaggtcacatgcgtggtggtggacgtgagccacgaagaccctgaggtcaagttcaactggtacgtggacggcgtggaggtgcataatgccaagacaaagccgcgggaggagcagtacaacagcacgtaccgtgtggtcagcgtcctcaccgtcctgcaccaggactggctgaatggcaaggagtacaagtgcaaggtctccaacaaagccctcccagcccccatcgagaaaaccatctccaaagccaaagggcagccccgagaaccacaggtgtacaccctgcccccatcccgggatgagctgaccaagaaccaggtcagcctgacctgcctggtcaaaggcttctatcccagcgacatcgccgtggagtgggagagcaatgggcagccggagaacaactacaagaccacgcctcccgtgttggactccgacggctccttcttcctctacagcaagctcaccgtggacaagagcaggtggcagcaggggaacgtcttctcatgctccgtgatgcatgaggctctgcacaaccactacacgcagaagagcctctccctgtctccgggtaaa